European Patent Application EP 4 714 970 A1, published March 25, 2026. Title: BISPECIFIC ANTIBODY, PHARMACEUTICAL COMPOSITION, AND USE. Applicant: Akeso Biopharma Co., Ltd. Application WO PCT/CN2024/084904, filed March 29, 2024. The sequence listing filed with the application follows.

SEQUENCE LISTING (62 sequences)

SEQ ID NO: 1 - protein, 360 aa, synthetic construct
CAGGTGCAGCTGCAGCAGTGGGGAGCTGGACTGCTGAAACCTAGCGAGACACTGAGCCTGACCTGTGCTGTGTACGGCGGATCTATCAGCGATTACTACTGGAACTGGATCAGGCAGCCCCCTGGAAAGGGACTGGAATGGATCGGAGAGATCAACTACAGGGGCACCACCAACTCCAATCCCTCTCTGAAGAGCAGGGTGACACTGAGCCTCGACACAAGCAAGAATCAGTTCAGCCTGAAGCTGAGGTCCGTGACCGCTGCTGATACAGCTGTGTACTACTGTGCCTTCGGCTACAGCGATTACGAGTACGATTGGTTCGACCCTTGGGGCCAGGGAACACTGGTTACAGTGAGCTCC

SEQ ID NO: 2 - protein, 120 aa, synthetic construct
QVQLQQWGAGLLKPSETLSLTCAVYGGSISDYYWNWIRQPPGKGLEWIGEINYRGTTNSNPSLKSRVTLSLDTSKNQFSLKLRSVTAADTAVYYCAFGYSDYEYDWFDPWGQGTLVTVSS

SEQ ID NO: 3 - DNA, 321 bp, synthetic construct
  source 1..321: mol_type = other DNA
gagatcgttctgacccagagcccagctacactgagcctgtctcctggagagagggctacactgtcctgcagagctagccagaccatcagcagctacctggcttggtaccagcagaagcctggccaagctccaaggctgctgatctacgacgcctctaatagggccaccggcatccctgctagattctctggaagcggcagcggaaccgactttacactgacaatcagctccctggagcccgaggatttcgctgtttactactgtcagcagcgcagcaactggcccatcacattcggacagggcacaaatctggagatcaag

SEQ ID NO: 4 - protein, 107 aa, synthetic construct
EIVLTQSPATLSLSPGERATLSCRASQTISSYLAWYQQKPGQAPRLLIYDASNRATGIPARFSGSGSGTDFTLTISSLEPEDFAVYYCQQRSNWPITFGQGTNLEIK

SEQ ID NO: 5 - DNA, 321 bp, synthetic construct
  source 1..321: mol_type = other DNA
gagatcgttctgacccagagcccagctacactgagcctgtctcctggagagagggctacactgtcctgcagagctagccagaccatcagcagctacctggcttggtaccagcagaagcctggccaagctccaaggctgctgatctacgacggctctaatagggccaccggcatccctgctagattctctggaagcggcagcggaaccgactttacactgacaatcagctccctggagcccgaggatttcgctgtttactactgtcagcagcgcagcaactggcccctcacattcggacagggcacaaatctggagatcaag

SEQ ID NO: 6 - protein, 107 aa, synthetic construct
EIVLTQSPATLSLSPGERATLSCRASQTISSYLAWYQQKPGQAPRLLIYDGSNRATGIPARFSGSGSGTDFTLTISSLEPEDFAVYYCQQRSNWPLTFGQGTNLEIK

SEQ ID NO: 7 - DNA, 321 bp, synthetic construct
  source 1..321: mol_type = other DNA
gagatcgttctgacccagagcccagctacactgagcctgtctcctggagagagggctacactgtcctgcagagctagccagtccatcagcagctacctggcttggtaccagcagaagcctggccaagctccaaggctgctgatctacgacggctctaatagggccaccggcatccctgctagattctctggaagcggcagcggaaccgactttacactgacaatcagctccctggagcccgaggatttcgctgtttactactgtcagcagcgcagcaactggcccatcacattcggacagggcacaaatctggagatcaag

SEQ ID NO: 8 - protein, 107 aa, synthetic construct
EIVLTQSPATLSLSPGERATLSCRASQSISSYLAWYQQKPGQAPRLLIYDGSNRATGIPARFSGSGSGTDFTLTISSLEPEDFAVYYCQQRSNWPITFGQGTNLEIK

SEQ ID NO: 9 - protein, 8 aa, synthetic construct
GGSISDYY

SEQ ID NO: 10 - protein, 7 aa, synthetic construct
INYRGTT

SEQ ID NO: 11 - protein, 14 aa, synthetic construct
AFGYSDYEYDWFDP

SEQ ID NO: 12 - protein, 6 aa, synthetic construct
QTISSY

SEQ ID NO: 13 - skipped

SEQ ID NO: 14 - protein, 9 aa, synthetic construct
QQRSNWPIT

SEQ ID NO: 15 - skipped

SEQ ID NO: 16 - protein, 9 aa, synthetic construct
QQRSNWPLT

SEQ ID NO: 17 - protein, 6 aa, synthetic construct
QSISSY

SEQ ID NO: 18 - protein, 330 aa, synthetic construct [sequence omitted]

SEQ ID NO: 19 - protein, 107 aa, synthetic construct [sequence omitted]

SEQ ID NO: 20 - protein, 327 aa, synthetic construct
ASTKGPSVFPLAPCSRSTSESTAALGCLVKDYFPEPVTVSWNSGALTSGVHTFPAVLQSSGLYSLSSVVTVPSSSLGTKTYTCNVDHKPSNTKVDKRVESKYGPPCPPCPAPEFLGGPSVFLFPPKPKDTLMISRTPEVTCVVVDVSQEDPEVQFNWYVDGVEVHNAKTKPREEQFNSTYRVVSVLTVLHQDWLNGKEYKCKVSNKGLPSSIEKTISKAKGQPREPQVYTLPPSQEEMTKNQVSLTCLVKGFYPSDIAVEWESNGQPENNYKTTPPVLDSDGSFFLYSRLTVDKSRWQEGNVFSCSVMHEALHNHYTQKSLSLSLGK

SEQ ID NO: 21 - protein, 448 aa, synthetic construct
EVQLVESGGGLVQPGGSLRLSCAASGFAFSSYDMSWVRQAPGKGLDWVATISGGGRYTYYPDSVKGRFTISRDNSKNNLYLQMNSLRAEDTALYYCANRYGEAWFAYWGQGTLVTVSSASTKGPSVFPLAPSSKSTSGGTAALGCLVKDYFPEPVTVSWNSGALTSGVHTFPAVLQSSGLYSLSSVVTVPSSSLGTQTYICNVNHKPSNTKVDKKVEPKSCDKTHTCPPCPAPEAAGAPSVFLFPPKPKDTLMISRTPEVTCVVVDVSHEDPEVKFNWYVDGVEVHNAKTKPREEQYNSTYRVVSVLTVLHQDWLNGKEYKCKVSNKALPAPIEKTISKAKGQPREPQVYTLPPSRDELTKNQVSLTCLVKGFYPSDIAVEWESNGQPENNYKTTPPVLDSDGSFFLYSKLTVDKSRWQQGNVFSCSVMHEALHNHYTQKSLSLSPGK

SEQ ID NO: 22 - protein, 214 aa, synthetic construct
DIQMTQSPSSMSASVGDRVTFTCRASQDINTYLSWFQQKPGKSPKTLIYRANRLVSGVPSRFSGSGSGQDYTLTISSLQPEDMATYYCLQYDEFPLTFGAGTKLELKRTVAAPSVFIFPPSDEQLKSGTASVVCLLNNFYPREAKVQWKVDNALQSGNSQESVTEQDSKDSTYSLSSTLTLSKADYEKHKVYACEVTHQGLSSPVTKSFNRGEC

SEQ ID NO: 23 - protein, 447 aa, synthetic construct
QVQLQQWGAGLLKPSETLSLTCAVYGGSFSDYYWNWIRQPPGKGLEWIGEINHRGSTNSNPSLKSRVTLSLDTSKNQFSLKLRSVTAADTAVYYCAFGYSDYEYNWFDPWGQGTLVTVSSASTKGPSVFPLAPCSRSTSESTAALGCLVKDYFPEPVTVSWNSGALTSGVHTFPAVLQSSGLYSLSSVVTVPSSSLGTKTYTCNVDHKPSNTKVDKRVESKYGPPCPPCPAPEFLGGPSVFLFPPKPKDTLMISRTPEVTCVVVDVSQEDPEVQFNWYVDGVEVHNAKTKPREEQFNSTYRVVSVLTVLHQDWLNGKEYKCKVSNKGLPSSIEKTISKAKGQPREPQVYTLPPSQEEMTKNQVSLTCLVKGFYPSDIAVEWESNGQPENNYKTTPPVLDSDGSFFLYSRLTVDKSRWQEGNVFSCSVMHEALHNHYTQKSLSLSLGK

SEQ ID NO: 24 - protein, 214 aa, synthetic construct
EIVLTQSPATLSLSPGERATLSCRASQSISSYLAWYQQKPGQAPRLLIYDASNRATGIPARFSGSGSGTDFTLTISSLEPEDFAVYYCQQRSNWPLTFGQGTNLEIKRTVAAPSVFIFPPSDEQLKSGTASVVCLLNNFYPREAKVQWKVDNALQSGNSQESVTEQDSKDSTYSLSSTLTLSKADYEKHKVYACEVTHQGLSSPVTKSFNRGEC

SEQ ID NO: 25 - protein, 8 aa, synthetic construct
GYSFTGYT

SEQ ID NO: 26 - protein, 8 aa, synthetic construct
INPYNAGT

SEQ ID NO: 27 - protein, 14 aa, synthetic construct
ARSEYRYGGDYFDY

SEQ ID NO: 28 - protein, 12 aa, synthetic construct
QSLLNSSNQKNY

SEQ ID NO: 29 - skipped

SEQ ID NO: 30 - protein, 9 aa, synthetic construct
QQHYDTPYT

SEQ ID NO: 31 - protein, 121 aa, synthetic construct
EVQLQQSGPELVKPGASMRMSCKASGYSFTGYTMNWVKQSHGKNLEWIGLINPYNAGTSYNQKFKGKATLTVDKSSSTAYMELLSLTSEDSAVYYCARSEYRYGGDYFDYWGQGTTLTVSS

SEQ ID NO: 32 - protein, 113 aa, synthetic construct
DIVMTQSPSSLAMSVGQKVTMSCKSSQSLLNSSNQKNYLAWYQQKPGQSPKLLVYFASTRESGVPDRFIGSGSGTDFTLTISSVQAEDLADYFCQQHYDTPYTFGGGTKLEIK

SEQ ID NO: 33 - protein, 121 aa, synthetic construct
QVQLQQSGAEVVKPGASMKMSCKASGYSFTGYTMNWVKQAHGQNLEWIGLINPYNAGTSYNQKFQGKATLTVDKSTSTAYMELSSLRSEDTAVYYCARSEYRYGGDYFDYWGQGTTLTVSS

SEQ ID NO: 34 - protein, 113 aa, synthetic construct
DIVMTQSPSSLAMSVGERVTMSCKSSQSLLNSSNQKNYLAWYQQKPGQAPKLLVYFASTRESGVPDRFSGSGSGTDFTLTISSVQAEDLADYFCQQHYDTPYTFGGGTKLEIK

SEQ ID NO: 35 - protein, 121 aa, synthetic construct
QVQLVQSGAEVVKPGASVKVSCKASGYSFTGYTMNWVRQAPGQNLEWIGLINPYNAGTSYNQKFQGKVTLTVDKSTSTAYMELSSLRSEDTAVYYCARSEYRYGGDYFDYWGQGTTLTVSS

SEQ ID NO: 36 - protein, 113 aa, synthetic construct
DIVMTQSPSSLAVSVGERVTISCKSSQSLLNSSNQKNYLAWYQQKPGQAPKLLIYFASTRESGVPDRFSGSGSGTDFTLTISSVQAEDVADYYCQQHYDTPYTFGGGTKLEIK

SEQ ID NO: 37 - protein, 113 aa, synthetic construct
DIVMTQSPSSLAVSVGERVTISCKSSQSLLNSSNQKNYLAWYQQKPGQAPKLLIYFASTRESGVPDRFSGSGSGTDFTLTISSLQAEDVAVYYCQQHYDTPYTFGGGTKLEIK

SEQ ID NO: 38 - protein, 450 aa, synthetic construct
QVQLQQWGAGLLKPSETLSLTCAVYGGSISDYYWNWIRQPPGKGLEWIGEINYRGTTNSNPSLKSRVTLSLDTSKNQFSLKLRSVTAADTAVYYCAFGYSDYEYDWFDPWGQGTLVTVSSASTKGPSVFPLAPSSKSTSGGTAALGCLVKDYFPEPVTVSWNSGALTSGVHTFPAVLQSSGLYSLSSVVTVPSSSLGTQTYICNVNHKPSNTKVDKKVEPKSCDKTHTCPPCPAPELLGGPSVFLFPPKPKDTLMISRTPEVTCVVVDVSHEDPEVKFNWYVDGVEVHNAKTKPREEQYNSTYRVVSVLTVLHQDWLNGKEYKCKVSNKALPAPIEKTISKAKGQPREPQVYTLPPSRDELTKNQVSLTCLVKGFYPSDIAVEWESNGQPENNYKTTPPVLDSDGSFFLYSKLTVDKSRWQQGNVFSCSVMHEALHNHYTQKSLSLSPGK

SEQ ID NO: 39 - protein, 214 aa, synthetic construct
EIVLTQSPATLSLSPGERATLSCRASQTISSYLAWYQQKPGQAPRLLIYDASNRATGIPARFSGSGSGTDFTLTISSLEPEDFAVYYCQQRSNWPITFGQGTNLEIKRTVAAPSVFIFPPSDEQLKSGTASVVCLLNNFYPREAKVQWKVDNALQSGNSQESVTEQDSKDSTYSLSSTLTLSKADYEKHKVYACEVTHQGLSSPVTKSFNRGEC

SEQ ID NO: 40 - protein, 451 aa, synthetic construct
QVQLVQSGAEVVKPGASVKVSCKASGYSFTGYTMNWVRQAPGQNLEWIGLINPYNAGTSYNQKFQGKVTLTVDKSTSTAYMELSSLRSEDTAVYYCARSEYRYGGDYFDYWGQGTTLTVSSASTKGPSVFPLAPSSKSTSGGTAALGCLVKDYFPEPVTVSWNSGALTSGVHTFPAVLQSSGLYSLSSVVTVPSSSLGTQTYICNVNHKPSNTKVDKKVEPKSCDKTHTCPPCPAPELLGGPSVFLFPPKPKDTLMISRTPEVTCVVVDVSHEDPEVKFNWYVDGVEVHNAKTKPREEQYNSTYRVVSVLTVLHQDWLNGKEYKCKVSNKALPAPIEKTISKAKGQPREPQVYTLPPSRDELTKNQVSLTCLVKGFYPSDIAVEWESNGQPENNYKTTPPVLDSDGSFFLYSKLTVDKSRWQQGNVFSCSVMHEALHNHYTQKSLSLSPGK

SEQ ID NO: 41 - protein, 220 aa, synthetic construct
DIVMTQSPSSLAVSVGERVTISCKSSQSLLNSSNQKNYLAWYQQKPGQAPKLLIYFASTRESGVPDRFSGSGSGTDFTLTISSLQAEDVAVYYCQQHYDTPYTFGGGTKLEIKRTVAAPSVFIFPPSDEQLKSGTASVVCLLNNFYPREAKVQWKVDNALQSGNSQESVTEQDSKDSTYSLSSTLTLSKADYEKHKVYACEVTHQGLSSPVTKSFNRGEC

SEQ ID NO: 42 - protein, 15 aa, synthetic construct
GGGGSGGGGSGGGGS

SEQ ID NO: 43 - protein, 20 aa, synthetic construct
GGGGSGGGGSGGGGSGGGGS

SEQ ID NO: 44 - protein, 120 aa, synthetic construct
QVQLQQWGAGLLKPSETLSLTCAVYGGSISDYYWNWIRQPPGKCLEWIGEINYRGTTNSNPSLKSRVTLSLDTSKNQFSLKLRSVTAADTAVYYCAFGYSDYEYDWFDPWGQGTLVTVSS

SEQ ID NO: 45 - protein, 107 aa, synthetic construct
EIVLTQSPATLSLSPGERATLSCRASQTISSYLAWYQQKPGQAPRLLIYDASNRATGIPARFSGSGSGTDFTLTISSLEPEDFAVYYCQQRSNWPITFGCGTNLEIK

SEQ ID NO: 46 - protein, 121 aa, synthetic construct
QVQLVQSGAEVVKPGASVKVSCKASGYSFTGYTMNWVRQAPGQCLEWIGLINPYNAGTSYNQKFQGKVTLTVDKSTSTAYMELSSLRSEDTAVYYCARSEYRYGGDYFDYWGQGTTLTVSS

SEQ ID NO: 47 - protein, 114 aa, synthetic construct
DIVMTQSPSSLAVSVGERVTISCKSSQSLLNSSNQKNYLAWYQQKPGQAPKLLIYFASTRESGVPDRFSGSGSGTDFTLTISSLQAEDVAVYYCQQHYDTPYTFGCGTKLEIKR

SEQ ID NO: 48 - protein, 5 aa, synthetic construct
GGGGS

SEQ ID NO: 49 - protein, 451 aa, synthetic construct
QVQLVQSGAEVVKPGASVKVSCKASGYSFTGYTMNWVRQAPGQNLEWIGLINPYNAGTSYNQKFQGKVTLTVDKSTSTAYMELSSLRSEDTAVYYCARSEYRYGGDYFDYWGQGTTLTVSSASTKGPSVFPLAPSSKSTSGGTAALGCLVKDYFPEPVTVSWNSGALTSGVHTFPAVLQSSGLYSLSSVVTVPSSSLGTQTYICNVNHKPSNTKVDKKVEPKSCDKTHTCPPCPAPEAAGGPSVFLFPPKPKDTLMISRTPEVTCVVVDVSHEDPEVKFNWYVDGVEVHNAKTKPREEQYNSTYRVVSVLTVLHQDWLNGKEYKCKVSNKALPAPIEKTISKAKGQPREPQVYTLPPSRDELTKNQVSLTCLVKGFYPSDIAVEWESNGQPENNYKTTPPVLDSDGSFFLYSKLTVDKSRWQQGNVFSCSVMHEALHNHYTQKSLSLSPGK

SEQ ID NO: 50 - protein, 220 aa, synthetic construct; identical to SEQ ID NO: 41

SEQ ID NO: 51 - protein, 718 aa, synthetic construct
QVQLVQSGAEVVKPGASVKVSCKASGYSFTGYTMNWVRQAPGQNLEWIGLINPYNAGTSYNQKFQGKVTLTVDKSTSTAYMELSSLRSEDTAVYYCARSEYRYGGDYFDYWGQGTTLTVSSASTKGPSVFPLAPSSKSTSGGTAALGCLVKDYFPEPVTVSWNSGALTSGVHTFPAVLQSSGLYSLSSVVTVPSSSLGTQTYICNVNHKPSNTKVDKKVEPKSCDKTHTCPPCPAPEAAGAPSVFLFPPKPKDTLMISRTPEVTCVVVDVSHEDPEVKFNWYVDGVEVHNAKTKPREEQYNSTYRVVSVLTVLHQDWLNGKEYKCKVSNKALPAPIEKTISKAKGQPREPQVYTLPPSRDELTKNQVSLTCLVKGFYPSDIAVEWESNGQPENNYKTTPPVLDSDGSFFLYSKLTVDKSRWQQGNVFSCSVMHEALHNHYTQKSLSLSPGKGGGGSGGGGSGGGGSGGGGSQVQLQQWGAGLLKPSETLSLTCAVYGGSISDYYWNWIRQPPGKCLEWIGEINYRGTTNSNPSLKSRVTLSLDTSKNQFSLKLRSVTAADTAVYYCAFGYSDYEYDWFDPWGQGTLVTVSSGGGGSGGGGSGGGGSGGGGSEIVLTQSPATLSLSPGERATLSCRASQTISSYLAWYQQKPGQAPRLLIYDASNRATGIPARFSGSGSGTDFTLTISSLEPEDFAVYYCQQRSNWPITFGCGTNLEIK

SEQ ID NO: 52 - protein, 713 aa, synthetic construct
QVQLVQSGAEVVKPGASVKVSCKASGYSFTGYTMNWVRQAPGQNLEWIGLINPYNAGTSYNQKFQGKVTLTVDKSTSTAYMELSSLRSEDTAVYYCARSEYRYGGDYFDYWGQGTTLTVSSASTKGPSVFPLAPSSKSTSGGTAALGCLVKDYFPEPVTVSWNSGALTSGVHTFPAVLQSSGLYSLSSVVTVPSSSLGTQTYICNVNHKPSNTKVDKKVEPKSCDKTHTCPPCPAPEAAGAPSVFLFPPKPKDTLMISRTPEVTCVVVDVSHEDPEVKFNWYVDGVEVHNAKTKPREEQYNSTYRVVSVLTVLHQDWLNGKEYKCKVSNKALPAPIEKTISKAKGQPREPQVYTLPPSRDELTKNQVSLTCLVKGFYPSDIAVEWESNGQPENNYKTTPPVLDSDGSFFLYSKLTVDKSRWQQGNVFSCSVMHEALHNHYTQKSLSLSPGKGGGGSGGGGSGGGGSQVQLQQWGAGLLKPSETLSLTCAVYGGSISDYYWNWIRQPPGKGLEWIGEINYRGTTNSNPSLKSRVTLSLDTSKNQFSLKLRSVTAADTAVYYCAFGYSDYEYDWFDPWGQGTLVTVSSGGGGSGGGGSGGGGSGGGGSEIVLTQSPATLSLSPGERATLSCRASQTISSYLAWYQQKPGQAPRLLIYDASNRATGIPARFSGSGSGTDFTLTISSLEPEDFAVYYCQQRSNWPITFGQGTNLEIK

SEQ ID NO: 53 - protein, 713 aa, synthetic construct
QVQLVQSGAEVVKPGASVKVSCKASGYSFTGYTMNWVRQAPGQNLEWIGLINPYNAGTSYNQKFQGKVTLTVDKSTSTAYMELSSLRSEDTAVYYCARSEYRYGGDYFDYWGQGTTLTVSSASTKGPSVFPLAPSSKSTSGGTAALGCLVKDYFPEPVTVSWNSGALTSGVHTFPAVLQSSGLYSLSSVVTVPSSSLGTQTYICNVNHKPSNTKVDKKVEPKSCDKTHTCPPCPAPEAAGAPSVFLFPPKPKDTLMISRTPEVTCVVVDVSHEDPEVKFNWYVDGVEVHNAKTKPREEQYNSTYRVVSVLTVLHQDWLNGKEYKCKVSNKALPAPIEKTISKAKGQPREPQVYTLPPSRDELTKNQVSLTCLVKGFYPSDIAVEWESNGQPENNYKTTPPVLDSDGSFFLYSKLTVDKSRWQQGNVFSCSVMHEALHNHYTQKSLSLSPGKGGGGSGGGGSGGGGSQVQLQQWGAGLLKPSETLSLTCAVYGGSISDYYWNWIRQPPGKCLEWIGEINYRGTTNSNPSLKSRVTLSLDTSKNQFSLKLRSVTAADTAVYYCAFGYSDYEYDWFDPWGQGTLVTVSSGGGGSGGGGSGGGGSGGGGSEIVLTQSPATLSLSPGERATLSCRASQTISSYLAWYQQKPGQAPRLLIYDASNRATGIPARFSGSGSGTDFTLTISSLEPEDFAVYYCQQRSNWPITFGCGTNLEIK

SEQ ID NO: 54 - protein, 725 aa, synthetic construct
QVQLQQWGAGLLKPSETLSLTCAVYGGSISDYYWNWIRQPPGKGLEWIGEINYRGTTNSNPSLKSRVTLSLDTSKNQFSLKLRSVTAADTAVYYCAFGYSDYEYDWFDPWGQGTLVTVSSASTKGPSVFPLAPSSKSTSGGTAALGCLVKDYFPEPVTVSWNSGALTSGVHTFPAVLQSSGLYSLSSVVTVPSSSLGTQTYICNVNHKPSNTKVDKKVEPKSCDKTHTCPPCPAPEAAGAPSVFLFPPKPKDTLMISRTPEVTCVVVDVSHEDPEVKFNWYVDGVEVHNAKTKPREEQYNSTYRVVSVLTVLHQDWLNGKEYKCKVSNKALPAPIEKTISKAKGQPREPQVYTLPPSRDELTKNQVSLTCLVKGFYPSDIAVEWESNGQPENNYKTTPPVLDSDGSFFLYSKLTVDKSRWQQGNVFSCSVMHEALHNHYTQKSLSLSPGKGGGGSGGGGSGGGGSGGGGSQVQLVQSGAEVVKPGASVKVSCKASGYSFTGYTMNWVRQAPGQNLEWIGLINPYNAGTSYNQKFQGKVTLTVDKSTSTAYMELSSLRSEDTAVYYCARSEYRYGGDYFDYWGQGTTLTVSSGGGGSGGGGSGGGGSGGGGSDIVMTQSPSSLAVSVGERVTISCKSSQSLLNSSNQKNYLAWYQQKPGQAPKLLIYFASTRESGVPDRFSGSGSGTDFTLTISSLQAEDVAVYYCQQHYDTPYTFGGGTKLEIKR

SEQ ID NO: 55 - protein, 725 aa, synthetic construct
QVQLQQWGAGLLKPSETLSLTCAVYGGSISDYYWNWIRQPPGKGLEWIGEINYRGTTNSNPSLKSRVTLSLDTSKNQFSLKLRSVTAADTAVYYCAFGYSDYEYDWFDPWGQGTLVTVSSASTKGPSVFPLAPSSKSTSGGTAALGCLVKDYFPEPVTVSWNSGALTSGVHTFPAVLQSSGLYSLSSVVTVPSSSLGTQTYICNVNHKPSNTKVDKKVEPKSCDKTHTCPPCPAPEAAGAPSVFLFPPKPKDTLMISRTPEVTCVVVDVSHEDPEVKFNWYVDGVEVHNAKTKPREEQYNSTYRVVSVLTVLHQDWLNGKEYKCKVSNKALPAPIEKTISKAKGQPREPQVYTLPPSRDELTKNQVSLTCLVKGFYPSDIAVEWESNGQPENNYKTTPPVLDSDGSFFLYSKLTVDKSRWQQGNVFSCSVMHEALHNHYTQKSLSLSPGKGGGGSGGGGSGGGGSGGGGSQVQLVQSGAEVVKPGASVKVSCKASGYSFTGYTMNWVRQAPGQCLEWIGLINPYNAGTSYNQKFQGKVTLTVDKSTSTAYMELSSLRSEDTAVYYCARSEYRYGGDYFDYWGQGTTLTVSSGGGGSGGGGSGGGGSGGGGSDIVMTQSPSSLAVSVGERVTISCKSSQSLLNSSNQKNYLAWYQQKPGQAPKLLIYFASTRESGVPDRFSGSGSGTDFTLTISSLQAEDVAVYYCQQHYDTPYTFGCGTKLEIKR

SEQ ID NO: 56 - protein, 447 aa, synthetic construct
EVQLLESGGGLVQPGGSLRLSCAASGFTFSSYAYSWVRQAPGKGLEWVSAISGSGGRTYYADSVKGRFTISRDNSKNTLYLQMNSLRAEDTAVYYCARLGYGRVDEWGRGTLVTVSSASTKGPSVFPLAPSSKSTSGGTAALGCLVKDYFPEPVTVSWNSGALTSGVHTFPAVLQSSGLYSLSSVVTVPSSSLGTQTYICNVNHKPSNTKVDKRVEPKSCDKTHTCPPCPAPEFEGGPSVFLFPPKPKDTLMISRTPEVTCVVVDVSHEDPEVKFNWYVDGVEVHNAKTKPREEQYNSTYRVVSVLTVLHQDWLNGKEYKCKVSNKALPASIEKTISKAKGQPREPQVYTLPPSREEMTKNQVSLTCLVKGFYPSDIAVEWESNGQPENNYKTTPPVLDSDGSFFLYSKLTVDKSRWQQGNVFSCSVMHEALHNHYTQKSLSLSPGK

SEQ ID NO: 57 - protein, 216 aa, synthetic construct
QSVLTQPPSASGTPGQRVTISCSGSLSNIGRNPVNWYQQLPGTAPKLLIYLDNLRLSGVPDRFSGSKSGTSASLAISGLQSEDEADYYCATWDDSHPGWTFGGGTKLTVLGQPKAAPSVTLFPPSSEELQANKATLVCLISDFYPGAVTVAWKADSSPVKAGVETTTPSKQSNNKYAASSYLSLTPEQWKSHRSYSCQVTHEGSTVEKTVAPTECS

SEQ ID NO: 58 - protein, 452 aa, synthetic construct
QVQLVQSGAEVEKPGASVKVSCKASGYTFTSYWITWVRQAPGQGLEWMGDIYPGSGNTNYNEKFKTRVTITADKSTSTAYMELSSLRSEDTAVYYCAKEGGLTTEDYALDYWGQGTLVTVSSASTKGPSVFPLAPSSKSTSGGTAALGCLVKDYFPEPVTVSWNSGALTSGVHTFPAVLQSSGLYSLSSVVTVPSSSLGTQTYICNVNHKPSNTKVDKKVEPKSCDKTHTCPPCPAPELLGGPSVFLFPPKPKDTLMISRTPEVTCVVVDVSHEDPEVKFNWYVDGVEVHNAKTKPREEQYQSTYRVVSVLTVLHQDWLNGKEYKCKVSNKALPAPIEKTISKAKGQPREPQVYTLPPSRDELTKNQVSLTCLVKGFYPSDIAVEWESNGQPENNYKTTPPVLDSDGSFFLYSKLTVDKSRWQQGNVFSCSVMHEALHNHYTQKSLSLSPGK

SEQ ID NO: 59 - protein, 218 aa, synthetic construct
EIVLTQSPATLSLSPGERATLSCRASKNVSTSGYSYMHWYQQKPGQAPRLLIYLASNLESGIPPRFSGSGYGTDFTLTINNIESEDAAYYFCQHSRELPFTFGQGTKVEIKRTVAAPSVFIFPPSDEQLKSGTASVVCLLNNFYPREAKVQWKVDNALQSGNSQESVTEQDSKDSTYSLSSTLTLSKADYEKHKVYACEVTHQGLSSPVTKSFNRGEC

SEQ ID NO: 60 - protein, 669 aa, synthetic construct
LQPGAEVPVVWAQEGAPAQLPCSPTIPLQDLSLLRRAGVTWQHQPDSGPPAAAPGHPLAPGPHPAAPSSWGPRPRRYTVLSVGPGGLRSGRLPLQPRVQLDERGRQRGDFSLWLRPARRADAGEYRAAVHLRDRALSCRLRLRLGQASMTASPPGSLRASDWVILNCSFSRPDRPASVHWFRNRGQGRVPVRESPHHHLAESFLFLPQVSPMDSGPWGCILTYRDGFNVSIMYNLTVLGLEPPTPLTVYAGAGSRVGLPCRLPAGVGTRSFLTAKWTPPGGGPDLLVTGDNGDFTLRLEDVSQAQAGTYTCHIHLQEQQLNATVTLAIITVTPKSFGSPGSLGKLLCEVTPVSGQERFVWSSLDTPSQRSFSGPWLEAQEAQLLSQPWQCQLYQGERLLGAAVYFTELSSPGAQRSGRAPGALPAGHLKLENLYFQGPRGPTIKPCPPCKCPAPNLLGGPSVFIFPPKIKDVLMISLSPIVTCVVVDVSEDDPDVQISWFVNNVEVHTAQTQTHREDYNSTLRVVSALPIQHQDWMSGKEFKCKVNNKDLPAPIERTISKPKGSVRAPQVYVLPPPEEEMTKKQVTLTCMVTDFMPEDIYVEWTNNGKTELNYKNTEPVLDSDGSYFMYSKLRVEKKNWVERNSYSCSVVHEGLHNHHTTKSFSRTPGK

SEQ ID NO: 61 - protein, 532 aa, synthetic construct
WELTILHTNDVHSRLEQTSEDSSKCVNASRCMGGVARLFTKVQQIRRAEPNVLLLDAGDQYQGTIWFTVYKGAEVAHFMNALRYDAMALGNHEFDNGVEGLIEPLLKEAKFPILSANIKAKGPLASQISGLYLPYKVLPVGDEVVGIVGYTSKETPFLSNPGTNLVFEDEITALQPEVDKLKTLNVNKIIALGHSGFEMDKLIAQKVRGVDVVVGGHSNTFLYTGNPPSKEVPAGKYPFIVTSDDGRKVPVVQAYAFGKYLGYLKIEFDERGNVISSHGNPILLNSSIPEDPSIKADINKWRIKLDNYSTQELGKTIVYLDGSSQSCRFRECNMGNLICDAMINNNLRHTDEMFWNHVSMCILNGGGIRSPIDERNNGTITWENLAAVLPFGGTFDLVQLKGSTLKKAFEHSVHRYGQSTGEFLQVGGIHVVYDLSRKPGDRVVKLDVLCTKCRVPSYDPLKMDEVYKVILPNFLANGGDGFQMIKDELLRHDSGDQDINVVSTYISKMKVIYPAVEGRIKFSTGSHHHHHH

SEQ ID NO: 62 - protein, 114 aa, synthetic construct
DIVMTQSPSSLAVSVGERVTISCKSSQSLLNSSNQKNYLAWYQQKPGQAPKLLIYFASTRESGVPDRFSGSGSGTDFTLTISSLQAEDVAVYYCQQHYDTPYTFGGGTKLEIKR